European Patent Application EP 4 714 977 A1, published March 25, 2026. Title: 활성화된 T세포의 선택적 제거용 항CD3 항체 및 이의 용도. Applicant: Seoul National University R&DB Foundation. The sequence listing filed with the application follows.

SEQUENCE LISTING (42 sequences)

SEQ ID NO: 1 - protein, 15 aa, synthetic construct
GGGGSGGGGSGGGGS

SEQ ID NO: 2 - protein, 107 aa, synthetic construct
RTVAAPSVFIFPPSDEQLKSGTASVVCLLNNFYPREAKVQWKVDNALQSGNSQESVTEQDSKDSTYSLSSTLTLSKADYEKHKVYACEVTHQGLSLPVTKSFNRGES

SEQ ID NO: 3 - protein, 10 aa, synthetic construct
YPYDVPDYAS

SEQ ID NO: 4 - protein, 6 aa, synthetic construct
HHHHHH

SEQ ID NO: 5 - protein, 10 aa, synthetic construct
SASSSVSYMN

SEQ ID NO: 6 - protein, 7 aa, synthetic construct
DTSKLAS

SEQ ID NO: 7 - protein, 9 aa, synthetic construct
QQWSSNPFT

SEQ ID NO: 8 - protein, 5 aa, synthetic construct
RYTMH

SEQ ID NO: 9 - protein, 17 aa, synthetic construct
YINPSRGYTNYNQKFKD

SEQ ID NO: 10 - protein, 10 aa, synthetic construct
YYDDHYCLDY

SEQ ID NO: 11 - protein, 107 aa, synthetic construct
QIVLTQSPAIMSASPGEKVTMTCSASSSVSYMNWYQQKSGTSPKRWIYDTSKLASGVPAHFRGSGSGTSYSLTISGMEAEDAATYYCQQWSSNPFTFGSGTKLEINR

SEQ ID NO: 12 - protein, 119 aa, synthetic construct [sequence omitted]

SEQ ID NO: 13 - protein, 241 aa, synthetic construct
QIVLTQSPAIMSASPGEKVTMTCSASSSVSYMNWYQQKSGTSPKRWIYDTSKLASGVPAHFRGSGSGTSYSLTISGMEAEDAATYYCQQWSSNPFTFGSGTKLEINRGGGGSGGGGSGGGGSQVQLQQSGAELARPGASVKMSCKASGYTFTRYTMHWVKQRPGQGLEWIGYINPSRGYTNYNQKFKDKATLTTDKSSSTAYMQLSSLTSEDSAVYYCARYYDDHYCLDYWGQGTTLTVSS

SEQ ID NO: 14 - protein, 11 aa, synthetic construct
RASQDIRNYLN

SEQ ID NO: 15 - protein, 7 aa, synthetic construct
YTSRLHS

SEQ ID NO: 16 - protein, 9 aa, synthetic construct
QQGNTLPWT

SEQ ID NO: 17 - protein, 10 aa, synthetic construct
GYSFTGYTMN

SEQ ID NO: 18 - protein, 10 aa, synthetic construct
LINPYKGVST

SEQ ID NO: 19 - protein, 13 aa, synthetic construct
SGYYGDSDWYFDV

SEQ ID NO: 20 - protein, 109 aa, synthetic construct
DIQMTQTTSSLSASLGDRVTISCRASQDIRNYLNWYQQKPDGTVKLLIYYTSRLHSGVPSKFSGSGSGTDYSLTISNLEQEDIATYFCQQGNTLPWTFAGGTKLEIKRA

SEQ ID NO: 21 - protein, 122 aa, synthetic construct
EVQLQQSGPELVKPGASMKISCKASGYSFTGYTMNWVKQSHGKNLEWMGLINPYKGVSTYNQKFKDKATLTVDKSSSTAYMELLSLTSEDSAVYYCARSGYYGDSDWYFDVWGAGTTVTVSS

SEQ ID NO: 22 - protein, 246 aa, synthetic construct
DIQMTQTTSSLSASLGDRVTISCRASQDIRNYLNWYQQKPDGTVKLLIYYTSRLHSGVPSKFSGSGSGTDYSLTISNLEQEDIATYFCQQGNTLPWTFAGGTKLEIKRAGGGGSGGGGSGGGGSEVQLQQSGPELVKPGASMKISCKASGYSFTGYTMNWVKQSHGKNLEWMGLINPYKGVSTYNQKFKDKATLTVDKSSSTAYMELLSLTSEDSAVYYCARSGYYGDSDWYFDVWGAGTTVTVSS

SEQ ID NO: 23 - protein, 8 aa, synthetic construct
SGSRYKYG

SEQ ID NO: 24 - protein, 7 aa, synthetic construct
NNDKRPS

SEQ ID NO: 25 - protein, 9 aa, synthetic construct
GNQDTSGAV

SEQ ID NO: 26 - protein, 8 aa, synthetic construct
GFSIGGYG

SEQ ID NO: 27 - protein, 17 aa, synthetic construct
TISRTGGTTWYGSAVKG

SEQ ID NO: 28 - protein, 22 aa, synthetic construct
ITAVCSTRSCSSRTYTVGQIDA

SEQ ID NO: 29 - protein, 101 aa, synthetic construct
LTQPSSVSANLGGTVKLTCSGSRYKYGWFQQKSPGSAPVTVIYNNDKRPSDIPSRFSGSASGSTATLTITGVQADDEAVYYCGNQDTSGAVFGVGTTLTVL

SEQ ID NO: 30 - protein, 131 aa, synthetic construct
AVTLDESGGGLQTPGGTLSLVCKASGFSIGGYGMGWVRQAPGKGLEWVGTISRTGGTTWYGSAVKGRATISRDSGQSTVRLQLNNLRAEDTGTYYCARITAVCSTRSCSSRTYTVGQIDAWGHGTEVIVSS

SEQ ID NO: 31 - protein, 250 aa, synthetic construct
LTQPSSVSANLGGTVKLTCSGSRYKYGWFQQKSPGSAPVTVIYNNDKRPSDIPSRFSGSASGSTATLTITGVQADDEAVYYCGNQDTSGAVFGVGTTLTVLGQSSRSSGGGGSSGGGGSAVTLDESGGGLQTPGGTLSLVCKASGFSIGGYGMGWVRQAPGKGLEWVGTISRTGGTTWYGSAVKGRATISRDSGQSTVRLQLNNLRAEDTGTYYCARITAVCSTRSCSSRTYTVGQIDAWGHGTEVIVSS

SEQ ID NO: 32 - protein, 8 aa, synthetic construct
SGGSSYYG

SEQ ID NO: 33 - protein, 7 aa, synthetic construct
ENDKRPS

SEQ ID NO: 34 - protein, 10 aa, synthetic construct
GTYDSNYVGI

SEQ ID NO: 35 - protein, 8 aa, synthetic construct
GFTFNSYD

SEQ ID NO: 36 - protein, 17 aa, synthetic construct
DINSRSSKTAYGAAVKG

SEQ ID NO: 37 - protein, 17 aa, synthetic construct
SASGGSNWPGAPASIDT

SEQ ID NO: 38 - protein, 102 aa, synthetic construct
LTQPSSVSANLGETVKITCSGGSSYYGWFQQKSPGSAPVTVIYENDKRPSDIPSRFSGSKSGSTGTLTITGVQADDEAVYFCGTYDSNYVGIFGAGTTLTVL

SEQ ID NO: 39 - protein, 126 aa, synthetic construct
AVTLDESGGGLQTPGGALSLVCKASGFTFNSYDMGWVRQAPGKGLEFVADINSRSSKTAYGAAVKGRATISRDNGQSTVRLQLNNLRAEDTATYYCAKSASGGSNWPGAPASIDTWGHGTEVIVSS

SEQ ID NO: 40 - protein, 246 aa, synthetic construct
LTQPSSVSANLGETVKITCSGGSSYYGWFQQKSPGSAPVTVIYENDKRPSDIPSRFSGSKSGSTGTLTITGVQADDEAVYFCGTYDSNYVGIFGAGTTLTVLGQSLRSSGGGGSSGGGGSAVTLDESGGGLQTPGGALSLVCKASGFTFNSYDMGWVRQAPGKGLEFVADINSRSSKTAYGAAVKGRATISRDNGQSTVRLQLNNLRAEDTATYYCAKSASGGSNWPGAPASIDTWGHGTEVIVSS

SEQ ID NO: 41 - protein, 221 aa, synthetic construct
QVQLQQSGAELARPGASVKMSCKASGYTFTRYTMHWVKQRPGQGLEWIGYINPSRGYTNYNQKFKDKATLTTDKSSSTAYMQLSSLTSEDSAVYYCARYYDDHYCLDYWGQGTTLTVSSAKTTPPSVYPLAPGSAAQTNSMVTLGCLVKGYFPEPVTVTWNSGSLSSGVHTFPAVLQSDLYTLSSSVTVPSSPRPSETVTCNVAHPASSTKVDKKIVPRDC

SEQ ID NO: 42 - protein, 213 aa, synthetic construct
QIVLTQSPAIMSASPGEKVTMTCSASSSVSYMNWYQQKSGTSPKRWIYDTSKLASGVPAHFRGSGSGTSYSLTISGMEAEDAATYYCQQWSSNPFTFGSGTKLEINRADAAPTVSIFPPSSEQLTSGGASVVCFLNNFYPKDINVKWKIDGSERQNGVLNSWTDQDSKDSTYSMSSTLTLTKDEYERHNSYTCEATHKTSTSPIVKSFNRNEC